European Patent Specification EP 4 329 780 B1, published November 26, 2025. Title: T CELL RECEPTORS DIRECTED AGAINST RAS-DERIVED RECURRENT NEOANTIGENS AND METHODS OF IDENTIFYING SAME. Applicant: Yeda Research And Development Co. Ltd. SAMUELS, Yardena FRIEDMAN, Nir PERI, Aviyah GREENSTEIN, Erez ALON, Michal. The sequence listing filed with the application follows.

SEQUENCE LISTING (40 sequences)

SEQ ID NO: 1 - protein, 10 aa, Artificial sequence
  neopeptide amino acid sequence
ILDTAGKEEY

SEQ ID NO: 2 - protein, 16 aa, Artificial sequence
  cdr3s Amino acid Sequence
CALSESHNNAGNMLTF

SEQ ID NO: 3 - protein, 11 aa, Artificial sequence
  cdr3s Amino acid Sequence
CAASQNTEAFF

SEQ ID NO: 4 - protein, 11 aa, Artificial sequence
  cdr3s Amino acid Sequence
CATDCKNQFYF

SEQ ID NO: 5 - protein, 17 aa, Artificial sequence
  cdr3s Amino acid Sequence
CASSLVSTPLPKETQYF

SEQ ID NO: 6 - protein, 12 aa, Artificial sequence
  cdr3s Amino acid Sequence
CALGDTAGKSTF

SEQ ID NO: 7 - protein, 17 aa, Artificial sequence
  cdr3s Amino acid Sequence
CASSLVSTPLPKETQYF

SEQ ID NO: 8 - protein, 13 aa, Artificial sequence
  cdr3s Amino acid Sequence
CAESSGGGFKTIF

SEQ ID NO: 9 - protein, 15 aa, Artificial sequence
  cdr3s Amino acid Sequence
CASSTPGPSAYEQYF

SEQ ID NO: 10 - protein, 14 aa, Artificial sequence
  cdr3s Amino acid Sequence
CALFGGTSYGKLTF

SEQ ID NO: 11 - protein, 11 aa, Artificial sequence
  cdr3s Amino acid Sequence
CAEGENTEAFF

SEQ ID NO: 12 - protein, 16 aa, Artificial sequence
  cdr3s Amino acid Sequence
CALSESGDAAGNKLTF

SEQ ID NO: 13 - protein, 11 aa, Artificial sequence
  cdr3s Amino acid Sequence
CAEGENTEAFF

SEQ ID NO: 14 - protein, 13 aa, Artificial sequence
  cdr3s Amino acid Sequence
CAEIPGGSYIPTF

SEQ ID NO: 15 - protein, 14 aa, Artificial sequence
  cdr3s Amino acid Sequence
CASSPWDIRTEAFF

SEQ ID NO: 16 - protein, 16 aa, Artificial sequence
  cdr3s Amino acid Sequence
CALSETINNAGNMLTF

SEQ ID NO: 17 - protein, 11 aa, Artificial sequence
  cdr3s Amino acid Sequence
CASSQNTEAFF

SEQ ID NO: 18 - DNA, 48 bp, Artificial sequence
  cdr3s nucleic acid sequence
tgtgctctgagtgagtcccataataatgcaggcaacatgctcaccttt

SEQ ID NO: 19 - DNA, 33 bp, Artificial sequence
  cdr3s nucleic acid sequence
tgtgccgcgagccagaacactgaagctttcttt

SEQ ID NO: 20 - DNA, 33 bp, Artificial sequence
  cdr3s nucleic acid sequence
tgtgctacggactgtaagaaccagttctatttt

SEQ ID NO: 21 - DNA, 51 bp, Artificial sequence
  cdr3s nucleic acid sequence
tgtgccagcagtttagtgtcaacaccactacctaaagagacccagtacttc

SEQ ID NO: 22 - DNA, 37 bp, Artificial sequence
  cdr3s nucleic acid sequence
tgtgctcttggggataccgcaggcaaatcaacctttg

SEQ ID NO: 23 - DNA, 51 bp, Artificial sequence; identical to SEQ ID NO: 21
  cdr3s nucleic acid sequence

SEQ ID NO: 24 - DNA, 39 bp, Artificial sequence
  cdr3s nucleic acid sequence
tgtgcagagagtagcggtggaggcttcaaaactatcttt

SEQ ID NO: 25 - DNA, 45 bp, Artificial sequence
  cdr3s nucleic acid sequence
tgtgccagcagtacaccgggaccatcggcgtacgagcagtacttc

SEQ ID NO: 26 - DNA, 42 bp, Artificial sequence
  cdr3s nucleic acid sequence
tgtgctctatttggtggtactagctatggaaagctgacattt

SEQ ID NO: 27 - DNA, 33 bp, Artificial sequence
  cdr3s nucleic acid sequence
tgtgccgagggagaaaacactgaagctttcttt

SEQ ID NO: 28 - DNA, 48 bp, Artificial sequence
  cdr3s nucleic acid sequence
tgtgctctgagtgagtcgggggatgctgcaggcaacaagctaactttt

SEQ ID NO: 29 - DNA, 33 bp, Artificial sequence; identical to SEQ ID NO: 27
  cdr3s nucleic acid sequence

SEQ ID NO: 30 - DNA, 39 bp, Artificial sequence
  cdr3s nucleic acid sequence
tgtgcagagataccgggaggaagctacatacctacattt

SEQ ID NO: 31 - DNA, 42 bp, Artificial sequence
  cdr3s nucleic acid sequence
tgtgccagcagtccctgggacattcgaactgaagctttcttt

SEQ ID NO: 32 - DNA, 48 bp, Artificial sequence
  cdr3s nucleic acid sequence
tgtgctctgagtgagaccattaataatgcaggcaacatgctcaccttt

SEQ ID NO: 33 - DNA, 33 bp, Artificial sequence
  cdr3s nucleic acid sequence
tgtgccagcagccagaacactgaagctttcttt

SEQ ID NO: 34 - protein, 10 aa, Artificial sequence
  neopeptide amino acid sequence
ILDTAGREEY

SEQ ID NO: 35 - protein, 10 aa, Artificial Sequence
  synthetic peptide
ILDTAGQEEY

SEQ ID NO: 36 - DNA, 20 bp, Artificial Sequence
  Single strand DNA oligonucleotide
ttggagcaggtggtgttggg

SEQ ID NO: 37 - DNA, 21 bp, Artificial Sequence
  Single strand DNA oligonucleotide
gtatcaactgtccttgttggc

SEQ ID NO: 38 - DNA, 25 bp, Artificial Sequence
  Single strand DNA oligonucleotide
taaacttgtggtagttggagctggt

SEQ ID NO: 39 - DNA, 21 bp, Artificial Sequence
  Single strand DNA oligonucleotide
ttctttgctgatttttttcaa

SEQ ID NO: 40 - protein, 10 aa, Artificial Sequence
  synthetic peptide
  misc_feature (7)..(7): Xaa can be any naturally occurring amino acid
ILDTAGXEEY